European Patent Application EP 4 628 103 A1, published October 8, 2025. Title: 抗HER3抗体药物偶联物组合物及其医药用途. Applicant: 苏州盛迪亚生物医药有限公司. Application CN. The sequence listing filed with the application follows.

SEQUENCE LISTING (10 sequences)

SEQ ID NO: 1 - protein, 5 aa, synthetic construct
DYAMH

SEQ ID NO: 2 - protein, 17 aa, synthetic construct
GISWNSGSIGYADSVKG

SEQ ID NO: 3 - protein, 8 aa, synthetic construct
EGLPGLDY

SEQ ID NO: 4 - protein, 11 aa, synthetic construct
RASQHVGTYLN

SEQ ID NO: 5 - protein, 7 aa, synthetic construct
GAANLQS

SEQ ID NO: 6 - protein, 10 aa, synthetic construct
QQSYNTPPFS

SEQ ID NO: 7 - protein, 117 aa, synthetic construct
QVQLVQSGGGLVQPGRSLRLSCAASGFTFDDYAMHWVRQAPGKGLEWVSGISWNSGSIGYADSVKGRFTISRDNAKNSLYLQMNSLRAEDTALYYCAKEGLPGLDYWGQGTLVTVSS

SEQ ID NO: 8 - protein, 108 aa, synthetic construct
DIQMTQSPSSLSASIGDRATITCRASQHVGTYLNWYQQKPGKTPKLLISGAANLQSGVPSRFSGSGSGTDFTLTISSLQPEDFATYYCQQSYNTPPFSFGQGTKVEIK

SEQ ID NO: 9 - protein, 447 aa, synthetic construct
QVQLVQSGGGLVQPGRSLRLSCAASGFTFDDYAMHWVRQAPGKGLEWVSGISWNSGSIGYADSVKGRFTISRDNAKNSLYLQMNSLRAEDTALYYCAKEGLPGLDYWGQGTLVTVSSASTKGPSVFPLAPSSKSTSGGTAALGCLVKDYFPEPVTVSWNSGALTSGVHTFPAVLQSSGLYSLSSVVTVPSSSLGTQTYICNVNHKPSNTKVDKKVEPKSCDKTHTCPPCPAPELLGGPSVFLFPPKPKDTLMISRTPEVTCVVVDVSHEDPEVKFNWYVDGVEVHNAKTKPREEQYNSTYRVVSVLTVLHQDWLNGKEYKCKVSNKALPAPIEKTISKAKGQPREPQVYTLPPSRDELTKNQVSLTCLVKGFYPSDIAVEWESNGQPENNYKTTPPVLDSDGSFFLYSKLTVDKSRWQQGNVFSCSVMHEALHNHYTQKSLSLSPGK

SEQ ID NO: 10 - protein, 215 aa, synthetic construct
DIQMTQSPSSLSASIGDRATITCRASQHVGTYLNWYQQKPGKTPKLLISGAANLQSGVPSRFSGSGSGTDFTLTISSLQPEDFATYYCQQSYNTPPFSFGQGTKVEIKRTVAAPSVFIFPPSDEQLKSGTASVVCLLNNFYPREAKVQWKVDNALQSGNSQESVTEQDSKDSTYSLSSTLTLSKADYEKHKVYACEVTHQGLSSPVTKSFNRGEC